European Patent Application EP 4 455 277 A1, published October 30, 2024. Title: Rebaudioside production. Applicant: SAMYANG CORPORATION. The sequence listing filed with the application follows.

SEQUENCE LISTING (36 sequences)

SEQ ID NO: 1 - protein, 461 aa, synthetic construct
  REGION 1..461: note = TaUGT wild-type Glycosyltransferase
MDDGSSSSSSPLRVVICPWLAFGHLLPCLDIAERLASRGHRVSFVSTPRNIARLPPVRPAVAPLVDYVALPLPRVDGLPEGAESTNDVPHDKFELLRKAFDGLAAPFSEFLHAACAEGTGKRPDWLIVDSFHHWAAAAAVENKVPCVMLLLGAANVIATWARGVSEHAAAAVGKERSAAEAPSFETERRKLMITQNASGMTVAERYFLTLMRSNLVAIRSCAEWEPESVAALTTLAGKPVVTLGLLPPSPEGGRGISKQDAAVRWLDAQRDKSVVYVALGSEVPLRVEQVHELALGLELSGASFLWALRKPPGMPDAAVLPPGFEERTRGRGLVVTGWVPQISVLAHGAVAAFLTHCGWNSTIEGLLFGQPLIMLPISSDQGPNARLMEGRKVGMQVPRNESDGSFTREDVAATVQAVAMEEDGSRVFTANAKTMQEIVADSACHERCIDGFIQQLRSYKE

SEQ ID NO: 2 - DNA, 1383 bp, synthetic construct
  misc_feature 1..1383: note = TaUGT wild-type Glycosyltransferase
  source 1..1383: mol_type = other DNA
atggacgacgggtcttctagctctagcagtccgctgcgtgttgttatttgcccgtggctggcttttggacacctgcttccatgcttagacattgcggaaagattagccagccgtggacacagagtatccttcgtaagtacgccgcgtaatatagcacgtttacccccggtcagaccggcagttgcgccgctggtcgattacgtagcgctacctctgcccagagtggacggacttccggaaggggctgaatctacaaacgacgtgccccatgataagttcgagcttttacgtaaggctttcgacggtttggcagcgcccttcagcgaatttctacacgcagcgtgcgcggagggcacaggcaaaagaccagattggcttattgtggattccttccaccattgggctgcggctgcggcagtggaaaataaagtcccgtgcgtcatgttacttttaggtgcagccaacgtgatcgccacttgggcacgtggcgtgtcagagcatgcggccgccgcggttggaaaagaacgtagtgccgcagaagctccatcattcgaaaccgaacgtcgtaaactgatgataactcagaatgcatcaggtatgaccgtagcagagcgttatttcctgacacttatgagatcaaacttggttgccattcgttcctgtgcagaatgggagcctgaatctgtggcggcactaaccactctggccgggaagcccgtagtgaccttaggtttgcttccaccgtctcctgagggaggaaggggtatttccaagcaagacgctgccgttaggtggctggacgctcagagggataagtccgttgtatacgtggcgttagggtctgaagttcccttgagagtggagcaggtacatgagcttgcgcttggactagagttgtcaggtgctagcttcctgtgggcgttacgtaagccacccggcatgcctgacgccgcagtcttgccgccgggttttgaagagagaaccaggggacgtggtctggttgtgactggctgggtaccacaaatcagcgtcttagcacatggcgccgttgccgcttttctgacacattgcggctggaatagtacaatcgaaggcttgctgttcggacaaccgttaatcatgctgccaatcagtagcgatcagggcccgaatgcccgtcttatggagggaagaaaagttggaatgcaggtgcctcgtaatgagtccgatggatcattcacaagagaggatgtcgctgccacagtacaagcagtagcgatggaggaggatgggagccgtgtttttacggctaatgcaaagaccatgcaagaaatagttgctgactccgcgtgtcacgaaaggtgcatcgatggatttatccaacagctaaggtcctataaagaa

SEQ ID NO: 3 - protein, 461 aa, synthetic construct
  REGION 1..461: note = TaUGT mutant Glycosyltransferase
MDDGSSSSSSPLRVVICPWLAFGHLLPCLDIAERLASRGHRVSFVSTPRNIARLPPVRPAVAPLVDYVALPLPRVDGLPEGAESTNDVPHDKFELLRKAFDGLAAPFSEFLHAACAEGTGKRPDWLIVDSFHHWAAAAAVENKVPCVMLLLGAANVIATWARGVSEHAAAAVGKERSAAEAPSFETERRKLMITQNASGMSLAERYFLTLMRSNLVAIRSCAEWEPESVAALTTLAGKPVVTLGLLPPSPEGGRGISKQDAAVRWLDAQRDKSVVYVALGSEVPLRVEQVHELALGLELSGASFLWALRKPPGMPDAAVLPPGFEERTRGRGLVVTGWVPQISVLAHGAVAAFLTHCGWNSTIEGLLFGQPLIMLPISSDQGPNARLMEGRKVGMQVPRNESDGSFTREDVAATVQAVAMEEDGSRVFTANAKTMQEIVADSACHERCIDGFIQQLRSYKE

SEQ ID NO: 4 - protein, 808 aa, synthetic construct
  REGION 1..808: note = SUS(Arabidopsis thaliana SUS1)
MANAERMITRVHSQRERLNETLVSERNEVLALLSRVEAKGKGILQQNQIIAEFEALPEQTRKKLEGGPFFDLLKSTQEAIVLPPWVALAVRPRPGVWEYLRVNLHALVVEELQPAEFLHFKEELVDGVKNGNFTLELDFEPFNASIPRPTLHKYIGNGVDFLNRHLSAKLFHDKESLLPLLKFLRLHSHQGKNLMLSEKIQNLNTLQHTLRKAEEYLAELKSETLYEEFEAKFEEIGLERGWGDNAERVLDMIRLLLDLLEAPDPCTLETFLGRVPMVFNVVILSPHGYFAQDNVLGYPDTGGQVVYILDQVRALEIEMLQRIKQQGLNIKPRILILTRLLPDAVGTTCGERLERVYDSEYCDILRVPFRTEKGIVRKWISRFEVWPYLETYTEDAAVELSKELNGKPDLIIGNYSDGNLVASLLAHKLGVTQCTIAHALEKTKYPDSDIYWKKLDDKYHFSCQFTADIFAMNHTDFIITSTFQEIAGSKETVGQYESHTAFTLPGLYRVVHGIDVFDPKFNIVSPGADMSIYFPYTEEKRRLTKFHSEIEELLYSDVENKEHLCVLKDKKKPILFTMARLDRVKNLSGLVEWYGKNTRLRELANLVVVGGDRRKESKDNEEKAEMKKMYDLIEEYKLNGQFRWISSQMDRVRNGELYRYICDTKGAFVQPALYEAFGLTVVEAMTCGLPTFATCKGGPAEIIVHGKSGFHIDPYHGDQAADTLADFFTKCKEDPSHWDEISKGGLQRIEEKYTWQIYSQRLLTLTGVYGFWKHVSNLDRLEARRYLEMFYALKYRPLAQAVPLAQDD

SEQ ID NO: 5 - DNA, 2424 bp, synthetic construct
  misc_feature 1..2424: note = SUS(Arabidopsis thaliana SUS1)
  source 1..2424: mol_type = other DNA
atggctaacgccgaacgtatgatcacgagggtacactcccaacgtgaacgtttaaatgaaactttggtcagcgagcgtaacgaggttctagcactactttccagggtcgaagctaaggggaaggggatacttcagcaaaatcagataatcgcggagttcgaggctttaccggagcagaccagaaaaaagttagagggtggcccgttctttgatctacttaaatctacacaggaggctattgtgctgccaccttgggtcgccctggcagtcaggcctaggccaggcgtatgggagtaccttcgtgttaatttgcacgcattagtagtggaggaattacagcctgccgaatttctacactttaaagaggagttagtggacggtgtcaagaatggaaacttcacccttgagcttgatttcgaaccattcaatgccagcataccccgtcctacattacacaaatatattgggaacggggtcgactttctgaataggcatctatcagctaagttgttccatgacaaggaatcccttcttcctctattgaaatttttgagacttcacagtcatcaggggaagaacttgatgttaagcgagaaaatacaaaacttgaatacgttacaacatacgcttagaaaggcagaggagtatctggcggaactaaagagtgagactttgtacgaagagttcgaagccaagtttgaggaaataggtcttgaacgtgggtggggcgacaatgctgaacgtgtcctggatatgatacgtcttttactggacttattagaggcaccggacccatgtaccctagaaacattcttagggagggtacccatggttttcaacgttgtcattcttagtccgcatggatattttgcccaagataacgtgttaggataccccgacaccgggggacaagttgtttatattttagatcaagtaagagcattagagattgagatgttacaaagaattaaacagcagggtctgaacataaaaccaaggatcttaattttgactcgtcttcttcctgatgcagtggggacgacgtgcggagagaggctggaacgtgtctacgattcagaatattgtgatatcctgagagtgccctttagaacagaaaaaggaatcgtgcgtaagtggatcagtagatttgaagtctggccatatctggagacatacaccgaagatgcagcggtcgaacttagcaaagagctaaacgggaaacccgacctgataatcgggaactacagcgacgggaatttagttgccagtttacttgcccataagctgggagtgacacagtgcacgatagcccacgcccttgaaaagacgaagtatcccgattctgacatatattggaaaaaacttgatgacaaataccatttttcatgccaattcactgctgatatctttgcaatgaatcacacggatttcatcattacttccacatttcaagagatcgcaggcagcaaagagacagttggacaatatgagagtcatactgcattcacactacctggtctttatagagtcgtgcacggtatagacgtgtttgatcctaagttcaacatagtctcaccgggtgcggatatgtccatctactttccctacactgaggaaaagaggcgtttaaccaagtttcattcagagatagaagagttattatatagtgatgtggaaaataaagagcatctatgcgtgttaaaagacaagaagaaacctatcctattcacaatggccagacttgacagagtgaagaatctatccggcttggttgaatggtacggcaagaacacgcgtcttcgtgagctagcgaaccttgtcgtagtaggaggtgacagaagaaaggaatccaaagacaacgaagagaaagcggagatgaaaaagatgtacgatctaatcgaagaatacaaattaaatggtcagttccgttggatctcctctcagatggatagagtccgtaatggagaactatacagatatatatgcgacaccaaaggcgcgtttgtgcagccggcattgtacgaggcctttggtctgactgtcgtcgaggccatgacctgcggccttcctacattcgcgacctgcaaaggtggtccagctgagattattgtccatgggaaatctggattccacatagacccatatcatggtgaccaggccgctgatacacttgcagatttttttactaagtgtaaggaggacccttcacattgggatgaaatatccaaagggggactgcagcgtatcgaggagaaatatacctggcaaatatatagccaaaggctgttgaccctaacgggcgtttacgggttctggaagcacgtttccaatctagataggctagaggcgaggcgttacctggaaatgttttacgcgttgaaatacaggcctctagcacaagcagtaccactggcgcaggacgat

SEQ ID NO: 6 - protein, 1275 aa, synthetic construct
  REGION 1..1275: note = Amino acid sequence of fused protein
MDDGSSSSSSPLRVVICPWLAFGHLLPCLDIAERLASRGHRVSFVSTPRNIARLPPVRPAVAPLVDYVALPLPRVDGLPEGAESTNDVPHDKFELLRKAFDGLAAPFSEFLHAACAEGTGKRPDWLIVDSFHHWAAAAAVENKVPCVMLLLGAANVIATWARGVSEHAAAAVGKERSAAEAPSFETERRKLMITQNASGMSLAERYFLTLMRSNLVAIRSCAEWEPESVAALTTLAGKPVVTLGLLPPSPEGGRGISKQDAAVRWLDAQRDKSVVYVALGSEVPLRVEQVHELALGLELSGASFLWALRKPPGMPDAAVLPPGFEERTRGRGLVVTGWVPQISVLAHGAVAAFLTHCGWNSTIEGLLFGQPLIMLPISSDQGPNARLMEGRKVGMQVPRNESDGSFTREDVAATVQAVAMEEDGSRVFTANAKTMQEIVADSACHERCIDGFIQQLRSYKEGGGGSGMANAERMITRVHSQRERLNETLVSERNEVLALLSRVEAKGKGILQQNQIIAEFEALPEQTRKKLEGGPFFDLLKSTQEAIVLPPWVALAVRPRPGVWEYLRVNLHALVVEELQPAEFLHFKEELVDGVKNGNFTLELDFEPFNASIPRPTLHKYIGNGVDFLNRHLSAKLFHDKESLLPLLKFLRLHSHQGKNLMLSEKIQNLNTLQHTLRKAEEYLAELKSETLYEEFEAKFEEIGLERGWGDNAERVLDMIRLLLDLLEAPDPCTLETFLGRVPMVFNVVILSPHGYFAQDNVLGYPDTGGQVVYILDQVRALEIEMLQRIKQQGLNIKPRILILTRLLPDAVGTTCGERLERVYDSEYCDILRVPFRTEKGIVRKWISRFEVWPYLETYTEDAAVELSKELNGKPDLIIGNYSDGNLVASLLAHKLGVTQCTIAHALEKTKYPDSDIYWKKLDDKYHFSCQFTADIFAMNHTDFIITSTFQEIAGSKETVGQYESHTAFTLPGLYRVVHGIDVFDPKFNIVSPGADMSIYFPYTEEKRRLTKFHSEIEELLYSDVENKEHLCVLKDKKKPILFTMARLDRVKNLSGLVEWYGKNTRLRELANLVVVGGDRRKESKDNEEKAEMKKMYDLIEEYKLNGQFRWISSQMDRVRNGELYRYICDTKGAFVQPALYEAFGLTVVEAMTCGLPTFATCKGGPAEIIVHGKSGFHIDPYHGDQAADTLADFFTKCKEDPSHWDEISKGGLQRIEEKYTWQIYSQRLLTLTGVYGFWKHVSNLDRLEARRYLEMFYALKYRPLAQAVPLAQDD

SEQ ID NO: 7 - protein, 4 aa, synthetic construct
  REGION 1..4: note = Linker for fused protein
GGGS

SEQ ID NO: 8 - protein, 5 aa, synthetic construct
  REGION 1..5: note = Linker for fused protein
GGGGS

SEQ ID NO: 9 - protein, 9 aa, synthetic construct
  REGION 1..9: note = Linker for fused protein
GGGSGGGGS

SEQ ID NO: 10 - protein, 15 aa, synthetic construct
  REGION 1..15: note = Linker for fused protein
GGGGSGGGGSGGGGS

SEQ ID NO: 11 - protein, 12 aa, synthetic construct
  REGION 1..12: note = Linker for fused protein
GGGGPSPGGGGS

SEQ ID NO: 12 - protein, 462 aa, synthetic construct
  REGION 1..462: note = EUGT11 enzyme
MDSGYSSSYAAAAGMHVVICPWLAFGHLLPCLDLAQRLASRGHRVSFVSTPRNISRLPPVRPALAPLVAFVALPLPRVEGLPDGAESTNDVPHDRPDMVELHRRAFDGLAAPFSEFLGTACADWVIVDVFHHWAAAAALEHKVPCAMMLLGSAHMIASIADRRLERAETESPAAAGQGRPAAAPTFEVARMKLIRTKGSSGMSLAERFSLTLSRSSLVVGRSCVEFEPETVPLLSTLRGKPITFLGLMPPLHEGRREDGEDATVRWLDAQPAKSVVYVALGSEVPLGVEKVHELALGLELAGTRFLWALRKPTGVSDADLLPAGFEERTRGRGVVATRWVPQMSILAHAAVGAFLTHCGWNSTIEGLMFGHPLIMLPIFGDQGPNARLIEAKNAGLQVARNDGDGSFDREGVAAAIRAVAVEEESSKVFQAKAKKLQEIVADMACHERYIDGFIQQLRSYKD

SEQ ID NO: 13 - DNA, 1386 bp, synthetic construct
  misc_feature 1..1386: note = EUGT11 enzyme
  source 1..1386: mol_type = other DNA
atggactccggctacagttcatcatatgctgcagccgctgggatgcacgttgtgatttgtccgtggctagcattcggtcatctgttgccgtgtttggacctggctcagaggctagcttccagaggacatcgtgtttccttcgtttctacgcctaggaatatcagtagactaccaccggtaagacctgctttagctccacttgtggcgttcgtggccctaccgttaccccgtgtagaaggattgcctgacggagcagagtctacgaatgacgtacctcacgacagacccgatatggttgaacttcacagaagagcgttcgacggtcttgctgcaccgttttccgaattccttgggacggcctgtgcggactgggtcatagtggacgtattccatcactgggctgccgcagctgccctagaacataaggttccgtgtgccatgatgttgttaggttctgctcatatgatcgcgtctattgcagaccgtaggttggagagggcagaaacggaaagtccagccgccgccggacaggggaggcccgctgcggcgccaacctttgaggtggctcgtatgaaactaattaggactaaaggttcaagcggtatgtcactggcggaaaggtttagtcttactttgtccaggtcttcattggtcgtcggtcgttcctgcgttgagtttgaacccgaaaccgttccccttctttccacgttacgtggaaaaccgattacttttcttggtcttatgccgccactgcacgagggtagaagggaagatggtgaagacgctacagttaggtggctagacgcgcaaccggctaagagcgtcgtctatgtcgcacttggctcagaggtgcccttgggggtcgagaaggtccatgagttggcgctggggttggagttggcgggtacaaggtttctttgggcccttcgtaaaccgacgggcgtatcagatgcagacctacttccggctggtttcgaggagcgtactaggggaaggggcgttgtggccacgagatgggtgccacaaatgagcatcctagctcatgccgcagtcggcgcattcttaacgcattgtggctggaattcaaccattgaagggctaatgttcggtcatccactgataatgcttcctatctttggagaccaaggtcccaatgcgcgtttgatcgaagccaagaatgctggccttcaagtcgcccgtaatgatggcgatggttcattcgacagagagggagtggcggcagcgatcagagcggttgcagtggaagaggagtccagtaaggtgtttcaggctaaggccaagaaattacaggagatagtggctgatatggcttgccacgagagatatatcgacggctttatacaacagctacgttcttataaggac

SEQ ID NO: 14 - protein, 463 aa, synthetic construct
  REGION 1..463: note = HvUGT enzyme
MDGDGNSSSSSSPLHVVICPWLALGHLLPCLDIAERLASRGHRVSFVSTPRNIARLPPLRPAVAPLVEFVALPLPHVDGLPEGAESTNDVPYDKFELHRKAFDGLAAPFSEFLRAACAEGAGSRPDWLIVDTFHHWAAAAAVENKVPCVMLLLGAATVIAGFARGVSEHAAAAVGKERPAAEAPSFETERRKLMTTQNASGMTVAERYFLTLMRSDLVAIRSCAEWEPESVAALTTLAGKPVVPLGLLPPSPEGGRGVSKEDAAVRWLDAQPAKSVVYVALGSEVPLRAEQVHELALGLELSGARFLWALRKPTDAPDAAVLPPGFEERTRGRGLVVTGWVPQIGVLAHGAVAAFLTHCGWNSTIEGLLFGHPLIMLPISSDQGPNARLMEGRKVGMQVPRDESDGSFRREDVAATVRAVAVEEDGRRVFTANAKKMQEIVADGACHERCIDGFIQQLRSYKA

SEQ ID NO: 15 - DNA, 1389 bp, synthetic construct
  misc_feature 1..1389: note = HvUGT enzyme
  source 1..1389: mol_type = other DNA
atggacggcgacggaaacagttcatcaagttctagtcctctgcatgttgttatatgtccctggctagctcttgggcatcttcttccttgtttggacattgcggaaagactggcctcaagaggacacagggtcagcttcgtatccacgccaagaaatattgcccgtctacccccgcttaggccagcggtggctcccttagtagagttcgttgctctacctctgcctcacgtggacgggttacctgaaggggctgaaagtacaaacgatgtaccctatgacaagtttgaacttcaccgtaaggcgttcgacgggctggccgctccttttagcgagttcttgagagctgcttgtgccgagggggctggttcccgtcctgattggctaatcgtggatacattccatcactgggcagcggcagccgccgttgaaaataaagtgccatgcgtgatgttactgcttggtgcagccaccgttattgccgggttcgcaagaggggtcagtgagcacgccgccgctgcagtcggtaaagagagaccggccgctgaagccccgagttttgagacggagagacgtaaacttatgaccactcagaatgcaagtggtatgacggttgcagaaaggtatttcctaaccttaatgcgtagtgacttggtcgcaatacgtagctgcgccgagtgggagcccgagtctgtcgcggcgttgacaaccttagcaggcaagcccgtcgttcctttaggcttgctgccaccgtctccagagggggggagaggcgtttccaaggaggacgccgcggttcgttggttggatgcgcaacccgcgaagagcgtcgtgtatgtcgcgttaggcagtgaggttccattgagagctgaacaagtccacgagttggcgcttggtttagaattatctggcgctaggtttttatgggcgctaaggaaacccaccgacgcgccagatgccgcggtattgccgccagggtttgaggaaaggactcgtggcagagggcttgtcgtgaccggttgggtgcctcaaatcggcgttcttgctcatggtgccgtagcagcattcttgactcattgtggctggaattcaaccatcgaggggctgctgtttggtcacccgttgatcatgctgccaataagctccgaccaaggacccaatgctcgtttgatggaaggcagaaaagtggggatgcaggtgcccagagacgaaagcgatgggagttttaggagagaagatgtggcagctactgttcgtgctgtagcggtggaggaagatggcagaagggtttttacagctaatgcgaagaagatgcaagaaatagtagccgacggggcttgtcacgagagatgcatcgatggatttatccaacaactgcgttcctacaaagct

SEQ ID NO: 16 - DNA, 28 bp, synthetic construct
  misc_feature 1..28: note = Reverse promoter of GAL10 promoter
  source 1..28: mol_type = other DNA
catcaattcttactttttttttggatgg

SEQ ID NO: 17 - DNA, 31 bp, synthetic construct
  misc_feature 1..31: note = Forward terminator of CYC1 terminator
  source 1..31: mol_type = other DNA
tgattgtcgatatcatgtaattagttatgtc

SEQ ID NO: 18 - DNA, 44 bp, synthetic construct
  misc_feature 1..44: note = Forward promoter of TaUGT connecting GAL10 promoter
  source 1..44: mol_type = other DNA
catccaaaaaaaaagtaagaattgatggacgacgggtcttctag

SEQ ID NO: 19 - DNA, 48 bp, synthetic construct
  misc_feature 1..48: note = Reverse promoter of TaUGT connecting CYC1 terminator
  source 1..48: mol_type = other DNA
ctaattacatgatatcgacaatcattctttataggaccttagctgttg

SEQ ID NO: 20 - DNA, 44 bp, synthetic construct
  misc_feature 1..44: note = Forward promoter of EUGT11 connecting GAL10 promoter
  source 1..44: mol_type = other DNA
catccaaaaaaaaagtaagaattgatggactccggctacagttc

SEQ ID NO: 21 - DNA, 45 bp, synthetic construct
  misc_feature 1..45: note = Reverse promoter of EUGT11 connecting CYC1 terminator
  source 1..45: mol_type = other DNA
ctaattacatgatatcgacaattagtccttataagaacgtagctg

SEQ ID NO: 22 - DNA, 42 bp, synthetic construct
  misc_feature 1..42: note = Forward promoter of HvUGT connecting GAL10 promoter
  source 1..42: mol_type = other DNA
catccaaaaaaaaagtaagaattgatggacggcgacggaaac

SEQ ID NO: 23 - DNA, 45 bp, synthetic construct
  misc_feature 1..45: note = Reverse promoter of HvUGT connecting CYC1 terminator
  source 1..45: mol_type = other DNA
ctaattacatgatatcgacaatcaagctttgtaggaacgcagttg

SEQ ID NO: 24 - DNA, 32 bp, synthetic construct
  misc_feature 1..32: note = Forward promoter for mutant T201S or V202L of TaUGT
  source 1..32: mol_type = other DNA
caggtatgtcwbtagcagagcgttatttcctg

SEQ ID NO: 25 - DNA, 34 bp, synthetic construct
  misc_feature 1..34: note = Reverse promoter for mutant T201S or V202L of TaUGT
  source 1..34: mol_type = other DNA
cgctctgctavwgacatacctgatgcattctgag

SEQ ID NO: 26 - DNA, 44 bp, synthetic construct; identical to SEQ ID NO: 18
  misc_feature 1..44: note = Forward promoter for mutant TaUGT
  source 1..44: mol_type = other DNA

SEQ ID NO: 27 - DNA, 43 bp, synthetic construct
  misc_feature 1..43: note = Reverse promoter for mutant TaUGT-LInker
  source 1..43: mol_type = other DNA
tccactaccaccgccaccttctttataggaccttagctgttgg

SEQ ID NO: 28 - DNA, 39 bp, synthetic construct
  misc_feature 1..39: note = Forward promoter for linker-SUS
  source 1..39: mol_type = other DNA
ggtggcggtggtagtggaatggctaacgccgaacgtatg

SEQ ID NO: 29 - DNA, 42 bp, synthetic construct
  misc_feature 1..42: note = Reverse promoter for SUS
  source 1..42: mol_type = other DNA
ctaattacatgatatcgacaattactcggcagccagagggac

SEQ ID NO: 30 - DNA, 1383 bp, synthetic construct
  misc_feature 1..1383: note = TaUGT mutant Glycosyltransferase
  source 1..1383: mol_type = other DNA
atggacgacgggtcttctagctctagcagtccgctgcgtgttgttatttgcccgtggctggcttttggacacctgcttccatgcttagacattgcagaaagattagccagccgtggacacagagtatccttcgtaagtacgccgcgtaatatagcacgtttacccccggtcagaccggcagttgcgccgctggtcgattacgtagcgctacctctgcccagagtggacggacttccggaaggggctgaatctacaaacgacgtgccccatgataagttcgagcttttacgtaaggctttcgacggtttggcagcgcccttcagcgaatttctacacgcagcgtgcgcggagggcacaggcaaaagaccagattggcttattgtggattccttccaccattgggctgcggctgcggcagtggaaaataaagtcccgtgcgtcatgttacttttaggtgcagccaacgtgatcgccacttgggcacgtggcgtgtcagagcatgcggccgccgcggttggaaaagaacgtagtgccgcagaagctccatcattcgaaaccgaacgtcgtaaactgatgataactcagaatgcatcaggtatgtcattagcagagcgttatttcctgacacttatgagatcaaacttggttgccattcgttcctgtgcagaatgggagcctgaatctgtggcggcactaaccactctggccgggaagcccgtagtgaccttaggtttgcttccaccgtctcctgagggaggaaggggtatttccaagcaagacgctgccgttaggtggctggacgctcagagggataagtccgttgtatacgtggcgttagggtctgaagttcccttgagagtggagcaggtacatgagcttgcgcttggactagagttgtcaggtgctagcttcctgtgggcgttacgtaagccacccggcatgcctgacgccgcagtcttgccgccgggttttgaagagagaaccaggggacgtggtctggttgtgactggctgggtaccacaaatcagcgtcttagcacatggcgccgttgccgcttttctgacacattgcggctggaatagtacaatcgaaggcttgctgttcggacaaccgttaatcatgctgccaatcagtagcgatcagggcccgaatgcccgtcttatggagggaagaaaagttggaatgcaggtgcctcgtaatgagtccgatggatcattcacaagagaggatgtcgctgccacagtacaagcagtagcgatggaggaggatgggagccgtgtttttacggctaatgcaaagaccatgcaagaaatagttgctgactccgcgtgtcacgaaaggtgcatcgatggatttatccaacagctaaggtcctataaagaa

SEQ ID NO: 31 - protein, 458 aa, synthetic construct
  REGION 1..458: note = SrUGT76G1_Protein
MENKTETTVRRRRRIILFPVPFQGHINPILQLANVLYSKGFSITIFHTNFNKPKTSNYPHFTFRFILDNDPQDERISNLPTHGPLAGMRIPIINEHGADELRRELELLMLASEEDEEVSCLITDALWYFAQSVADSLNLRRLVLMTSSLFNFHAHVSLPQFDELGYLDPDDKTRLEEQASGFPMLKVKDIKSAYSNWQILKEILGKMIKQTKASSGVIWNSFKELEESELETVIREIPAPSFLIPLPKHLTASSSSLLDHDRTVFQWLDQQPPSSVLYVSFGSTSEVDEKDFLEIARGLVDSKQSFLWVVRPGFVKGSTWVEPLPDGFLGERGRIVKWVPQQEVLAHGAIGAFWTHSGWNSTLESVCEGVPMIFSDFGLDQPLNARYMSDVLKVGVYLENGWERGEIANAIRRVMVDEEGEYIRQNARVLKQKADVSLMKGGSSYESLESLVSYISSL

SEQ ID NO: 32 - DNA, 1374 bp, synthetic construct
  misc_feature 1..1374: note = SrUGT76G1_DNA
  source 1..1374: mol_type = other DNA
atggaaaacaagacggaaaccactgttagaaggagaagaaggattatcttgttcccagttccattccaaggtcatattaatccaattttgcaattggctaatgtcttgtattctaaaggtttctctattactatattccatactaatttcaataaaccaaagacttctaattatccacatttcactttcagattcatattggataatgatccacaagatgaaagaatttctaatttgccaactcatggtccattggctggtatgagaattccaattattaatgaacatggtgctgatgaattgagaagagaattggaattgttgatgttggcttctgaagaagatgaggaagtttcttgtttgattactgatgctttgtggtatttcgctcaatctgttgctgattctttgaatttgagaagattggttttgatgacatcttctttgttcaatttccatgctcatgtttctttaccacaattcgatgaattgggttatttagatccagatgataagactagattggaagaacaagcttctggtttcccaatgttgaaagttaaagatattaaatctgcttattctaattggcaaatcttgaaagaaatcttgggtaagatgattaaacaaactaaagcttcttcaggtgttatttggaattctttcaaagaattggaagagtctgaattggaaactgttattagagaaattccagctccatctttcttgattccattgccaaaacatttgactgcttcatcttcctctttgttagatcatgatagaacagttttccaatggttggatcagcaaccaccatcttctgtcttgtatgtttctttcggttctacttctgaagttgatgagaaagatttcttggaaattgctagaggtttggttgattctaaacaatctttcttatgggttgttagaccaggtttcgttaaaggttctacatgggttgaaccattgccagatggtttcttgggtgaaagaggtagaattgttaaatgggttccacagcaagaagttttggctcatggtgctattggtgctttctggactcattctggttggaattctactttggaatctgtttgtgaaggtgttccaatgattttctctgatttcggtttggatcaaccattgaatgctagatatatgtctgatgtcttgaaagttggtgtttatttggaaaatggttgggaaagaggtgaaattgctaatgctattagaagagttatggttgatgaggaaggtgaatatattagacaaaatgctagagttttgaaacagaaagctgatgtttctttgatgaaaggtggttcttcttatgaatctttggaatctttggtatcctacatctcttccttg

SEQ ID NO: 33 - protein, 805 aa, synthetic construct
  REGION 1..805: note = Sucrose_synthase_Glycine max_Protein
MATDRLTRVHELRERLDETLTANRNEILALLSRIEAKGKGILQHHQVIAEFEEIPEENRQKLTDGAFGEVLRSTQEAIVLPPWVALAVRPRPGVWEYLRVNVHALVVEELQPAEYLHFKEELVDGSSNGNFVLELDFEPFNAAFPRPTLNKSIGNGVQFLNRHLLAKLFHDKESLHPLLEFLRLHSVKGKTLMLNDRIQNPDALQHVLRKAEEYLGTVPPETPYSEFEHKFQEIGLERGWGDNAERVLESIQLLLDLLEAPDPCTLETFLGRIPMVFNVVILSPHGYFAQDNVLGYPDTGGQVVYILDQVRALENEMLHRIKQQGLDIVPRILIITRLLPDAVGTTCGQRLEKVFGTEHSHILRVPFRTEKGIVRKWISRFEVWPYLETYTEDVAHELAKELQGKPDLIVGNYSDGNIVASLLAHKLGVTQCTIAHALEKTKYPESDIYWKKLEERYHFSCQFTADLFAMNHTDFIITSTFQEIAGSKDTVGQYESHTAFTLPGLYRVVHGIDVFDPKFNIVSPGADQTIYFPHTETSRRLTSFHPEIEELLYSSVENEEHICVLKDRSKPIIFTMARLDRVKNITGLVEWYGKNAKLRELVNLVVVAGDRRKESKDLEEKAEMKKMYGLIETYKLNGQFRWISSQMNRVRNGELYRVICDTRGAFVQPAVYEAFGLTVVEAMTCGLPTFATCNGGPAEIIVHGKSGFHIDPYHGDRAADLLVDFFEKCKLDPTHWDKISKAGLQRIEEKYTWQIYSQRLLTLTGVYGFWKHVSNLDRRESRRYLEMFYALKYRKLAESVPLAAE

SEQ ID NO: 34 - DNA, 2415 bp, synthetic construct
  misc_feature 1..2415: note = Sucrose_synthase_Glycine max_DNA
  source 1..2415: mol_type = other DNA
atggccacggacagactgactcgtgtacacgaattacgtgagaggttggacgagacgctaacagcaaacaggaacgagatactggcattgctttcaaggatagaagcaaagggtaagggaattctacagcatcaccaagtcatagcagaattcgaagaaatacctgaggagaatcgtcaaaagttaacagatggggccttcggagaagtcctaaggagtacacaagaggcaatagttctacctccgtgggtggcactagctgttagacctaggcctggagtctgggaatatctaagggtgaacgttcatgctctggttgtagaggaactacagccagcagaatatcttcacttcaaggaagaacttgttgacggctcatcaaatggcaatttcgtgttggaactggattttgagccgtttaacgccgctttcccgaggccgacgctaaataaaagtataggtaatggtgttcaatttcttaacaggcatcttctagccaaattgttccacgataaagagagtcttcaccccttattggaatttctacgtctacactctgttaagggcaagacattgatgttaaatgataggatacagaatccagacgcacttcagcatgttctgagaaaggccgaggaatacctaggaaccgtacccccggaaactccttactcagaattcgaacataagtttcaagagatcggtctagaaagaggatggggtgataacgctgaacgtgtattagagtctatacagcttttgcttgacttactagaagcgcctgacccctgcactctagaaacattcttgggaaggattccaatggtcttcaatgtcgtaatacttagtccacacgggtattttgctcaagataacgtacttggatatcctgacactgggggccaagtagtatacattctagaccaagtcagggctttggagaatgagatgctacacagaattaagcaacaaggtcttgacatagtacctcgtatattgataattactagattgctaccggatgccgttgggacgacgtgtgggcaacgtctagagaaagtgttcgggactgaacacagccatatcttgcgtgtaccgttcaggaccgaaaaagggattgtgcgtaaatggattagtagatttgaggtttggccgtacctagaaacgtatacggaagatgtcgcgcatgagttggctaaggagctgcaaggtaaacccgacttgatcgtcggtaactattccgacggtaacattgttgcgtcccttcttgcacataaactaggcgttacacagtgtactatcgctcatgccttggaaaaaacgaaatatcccgaatctgacatttactggaagaaattggaagagagatatcatttctcatgtcaattcacagcagaccttttcgctatgaaccacacggacttcattataacttctacatttcaagagatagcgggctcaaaggatactgttggccagtatgaaagtcatacggcttttacattgccgggcctgtatagggtcgtacatggcattgacgttttcgaccctaaattcaacatagtttccccaggtgcggaccagaccatttacttcccacacactgaaacctcaaggcgtttgacgtctttccatccagagatagaagaattactgtattcaagtgttgagaacgaagagcatatatgcgtacttaaggatcgttctaaaccaattatctttacgatggcgaggcttgatagagtcaagaatatcacgggccttgttgagtggtacgggaagaatgccaagctaagagagctggtgaatcttgtcgttgtcgctggagacagaagaaaggaaagtaaggaccttgaggagaaagcagagatgaagaaaatgtatggcttaatcgaaacatataaactaaatggtcagttcaggtggatatcaagtcagatgaaccgtgtacgtaatggcgaattatacagagtcatctgtgacactaggggtgctttcgtacagccggctgtatacgaggcttttggcctgacagtagtggaagccatgacgtgcggccttcctacgttcgcaacgtgtaacgggggaccagctgaaatcattgttcacggcaaaagcggattccacatagacccctaccacggcgatagagccgccgacttgttagtggatttcttcgagaaatgtaaactagaccctacccactgggacaaaatcagtaaagcaggattacaacgtattgaagaaaaatatacatggcaaatctactcacaacgtttgttaactttaaccggtgtgtatggtttttggaagcacgtgagcaaccttgacaggagagaaagcaggcgttacctggaaatgttctacgccttgaaatataggaaattggctgagtcagtccctctggctgccgag

SEQ ID NO: 35 - DNA, 446 bp, synthetic construct
  misc_feature 1..446: note = SUC2 upstream sequence 446-bp
  source 1..446: mol_type = other DNA
aaattatccgggggcgaagaaatacgcgtagcgttaatcgaccccacgtccagggtttttccatggaggtttctggaaaaactgacgaggaatgtgattataaatccctttatgtgatgtctaagacttttaaggtacgcccgatgtttgcctattaccatcatagagacgtttcttttcgaggaatgcttaaacgactttgtttgacaaaaatgttgcctaagggctctatagtaaaccatttggaagaaagatttgacgactttttttttttggatttcgatcctataatccttcctcctgaaaagaaacatataaatagatatgtattattcttcaaaacattctcttgttcttgtgctttttttttaccatatatcttacttttttttttctctcagagaaacaagcaaaacaaaaagcttttcttttcactaacgtatatg

SEQ ID NO: 36 - DNA, 358 bp, synthetic construct
  misc_feature 1..358: note = SUC2 downstream sequence 358-p
  source 1..358: mol_type = other DNA
ggttataaaacttattgtcttttttatttttttcaaaagccattctaaagggctttagctaacgagtgacgaatgtaaaactttatgatttcaaagaatacctccaaaccattgaaaatgtatttttatttttattttctcccgaccccagttacctggaatttgttctttatgtactttatataagtataattctcttaaaaatttttactactttgcaatagacatcattttttcacgtaataaacccacaatcgtaatgtagttgccttacactactaggatggacctttttgcctttatctgttttgttactgacacaatgaaaccgggtaaagtattagttatgtgaaaattt